European Patent Application EP 4 759 931 A1, published June 17, 2026. Title: Secretion signal petide gene derived from Hydrogenophilus bacterium. Applicant: 株式会社ＣＯ２資源化研究所. The sequence listing filed with the application follows.

SEQUENCE LISTING (181 sequences)

SEQ ID NO: 1 - protein, 27 aa, Hydrogenophilus thermoluteolus
MERRRFLKGAGLAGILAAGTAPAIIHA

SEQ ID NO: 2 - DNA, 81 bp, Hydrogenophilus thermoluteolus
  source 1..81: mol_type = genomic DNA
atggaacgtcgtcgtttcctcaaaggcgccggccttgccggcattctggctgccggcacggcgcctgcgatcatccatgca

SEQ ID NO: 3 - protein, 25 aa, Hydrogenophilus thermoluteolus
MTYRSQLVASLAAAGLIATSSAAFA

SEQ ID NO: 4 - DNA, 75 bp, Hydrogenophilus thermoluteolus
  source 1..75: mol_type = genomic DNA
atgacataccgttcccaactcgttgcttcactcgctgccgcggggctcatcgcaacttcgagcgccgcgtttgcc

SEQ ID NO: 5 - protein, 24 aa, Hydrogenophilus thermoluteolus
MKKPVLKSLTVALGVAFAAGAAWA

SEQ ID NO: 6 - DNA, 72 bp, Hydrogenophilus thermoluteolus
  source 1..72: mol_type = genomic DNA
atgaaaaaaccggtgctcaaatcgctgaccgttgcattgggcgttgcgttcgccgcaggtgctgcctgggcc

SEQ ID NO: 7 - protein, 25 aa, Hydrogenophilus thermoluteolus
MQRRTFLTALTAALIAAPVSATVAA

SEQ ID NO: 8 - DNA, 75 bp, Hydrogenophilus thermoluteolus
  source 1..75: mol_type = genomic DNA
atgcaacgccgaacgtttctgaccgcactcaccgcagcgctgatcgctgcgcccgtttcggcaaccgttgcggcc

SEQ ID NO: 9 - protein, 24 aa, Hydrogenophilus thermoluteolus
MKPMKWLTALAVTATVASAPVTHA

SEQ ID NO: 10 - DNA, 72 bp, Hydrogenophilus thermoluteolus
  source 1..72: mol_type = genomic DNA
atgaaacccatgaaatggctcaccgcattggcagtcaccgcaacggtggccagcgcgccggtcacccacgcg

SEQ ID NO: 11 - protein, 30 aa, Hydrogenophilus thermoluteolus
MNRMDRRIFLQGLGATVAVGAVGAPSLALG

SEQ ID NO: 12 - DNA, 90 bp, Hydrogenophilus thermoluteolus
  source 1..90: mol_type = genomic DNA
atgaatcggatggatcgtcggatattcttgcaaggcctgggcgcgaccgttgcagtcggagccgtgggtgcaccgtcgctcgcgttgggt

SEQ ID NO: 13 - protein, 24 aa, Hydrogenophilus thermoluteolus
MKRREFLHSSLAALLFLVAWHAQA

SEQ ID NO: 14 - DNA, 72 bp, Hydrogenophilus thermoluteolus
  source 1..72: mol_type = genomic DNA
atgaaaagacgggaatttctacacagttcactcgcagccctgttgtttctggttgcgtggcacgctcaagcg

SEQ ID NO: 15 - protein, 21 aa, Hydrogenophilus thermoluteolus
MKRKSFVSIVALAGFSPMILA

SEQ ID NO: 16 - DNA, 63 bp, Hydrogenophilus thermoluteolus
  source 1..63: mol_type = genomic DNA
atgaagcgtaaaagttttgtatcgatcgttgcgttggcgggtttttcgcccatgatcttagcc

SEQ ID NO: 17 - protein, 29 aa, Hydrogenophilus thermoluteolus
MMRMRSKWKKSAMVALAVTGLWGSGVGQA

SEQ ID NO: 18 - DNA, 87 bp, Hydrogenophilus thermoluteolus
  source 1..87: mol_type = genomic DNA
atgatgcgcatgcgcagcaaatggaagaaaagcgcgatggttgcgcttgcggtcacgggcctttggggtagcggcgtcgggcaggcg

SEQ ID NO: 19 - protein, 27 aa, Hydrogenophilus thermoluteolus
MKLRNTLSLVATLAVAGVVTTPAVTFA

SEQ ID NO: 20 - DNA, 81 bp, Hydrogenophilus thermoluteolus
  source 1..81: mol_type = genomic DNA
atgaaacttcgcaacaccctttccctggtcgccacgcttgccgtagcgggtgtcgtcacaaccccggcggtgaccttcgcg

SEQ ID NO: 21 - protein, 26 aa, Hydrogenophilus thermoluteolus
MAMNRREFLQVLAVAAAGGWSLTSNA

SEQ ID NO: 22 - DNA, 78 bp, Hydrogenophilus thermoluteolus
  source 1..78: mol_type = genomic DNA
atggcaatgaatcgacgtgaattcctgcaagtgctggcggttgcggcggctggcggctggagtctgaccagcaacgcc

SEQ ID NO: 23 - protein, 19 aa, Hydrogenophilus thermoluteolus
MKRIAMITALTLCAAAAHA

SEQ ID NO: 24 - DNA, 57 bp, Hydrogenophilus thermoluteolus
  source 1..57: mol_type = genomic DNA
atgaaacgcatcgccatgatcacagcgctcacactctgtgccgcagcagcacacgcc

SEQ ID NO: 25 - protein, 24 aa, Hydrogenophilus thermoluteolus
MKQKTLLAAVGAALAVAAVAPAQA

SEQ ID NO: 26 - DNA, 72 bp, Hydrogenophilus thermoluteolus
  source 1..72: mol_type = genomic DNA
atgaagcaaaaaacccttttggcagcggttggcgctgcattggcggttgcggcggtggcacccgcacaagcc

SEQ ID NO: 27 - protein, 27 aa, Hydrogenophilus thermoluteolus
MKTISQRMIRLTAASVFAGAFALPLWA

SEQ ID NO: 28 - DNA, 81 bp, Hydrogenophilus thermoluteolus
  source 1..81: mol_type = genomic DNA
atgaaaaccattagccagcgcatgatccgtttgaccgctgcatccgtctttgcgggtgccttcgcactccccctctgggct

SEQ ID NO: 29 - protein, 21 aa, Hydrogenophilus thermoluteolus
MKLKTVVFALAAIGVMGAAQA

SEQ ID NO: 30 - DNA, 63 bp, Hydrogenophilus thermoluteolus
  source 1..63: mol_type = genomic DNA
atgaaactgaagaccgttgtgtttgcattggctgcgatcggcgtgatgggcgcggcgcaagcg

SEQ ID NO: 31 - protein, 33 aa, Hydrogenophilus thermoluteolus
MHNDFGDLLTRRAWLRTAGGLLALAALPRAGIA

SEQ ID NO: 32 - DNA, 99 bp, Hydrogenophilus thermoluteolus
  source 1..99: mol_type = genomic DNA
atgcacaatgactttggtgatctgcttacccgtcgcgcgtggcttcgcaccgcaggcgggttgcttgcgttggctgcgctgccgcgtgccggcatagcc

SEQ ID NO: 33 - protein, 27 aa, Hydrogenophilus thermoluteolus
MVRRRAFLTGILGVTVLAIAPGSRVYA

SEQ ID NO: 34 - DNA, 81 bp, Hydrogenophilus thermoluteolus
  source 1..81: mol_type = genomic DNA
atggtgagacggcgtgcattcctcactgggatcttgggtgtgacggttttggcgattgcgccgggcagccgagtttatgcg

SEQ ID NO: 35 - protein, 24 aa, Hydrogenophilus thermoluteolus
MKKTVTAVALLCALSSTAIAPTFA

SEQ ID NO: 36 - DNA, 72 bp, Hydrogenophilus thermoluteolus
  source 1..72: mol_type = genomic DNA
atgaagaaaaccgtcacagctgttgcgcttctctgtgcgctgagcagcacggcgattgccccaacgtttgct

SEQ ID NO: 37 - protein, 18 aa, Hydrogenophilus thermoluteolus
MRVRFVLAGLLITGTVSA

SEQ ID NO: 38 - DNA, 54 bp, Hydrogenophilus thermoluteolus
  source 1..54: mol_type = genomic DNA
atgcgtgttcgcttcgttttggccggtttgctcatcaccggcacggtttccgct

SEQ ID NO: 39 - protein, 22 aa, Hydrogenophilus thermoluteolus
MKRWLSIAVFSVWFFGFGPAQA

SEQ ID NO: 40 - DNA, 66 bp, Hydrogenophilus thermoluteolus
  source 1..66: mol_type = genomic DNA
atgaagcgatggctatcgatcgcggttttttccgtgtggtttttcggtttcggcccggcgcaggct

SEQ ID NO: 41 - protein, 27 aa, Hydrogenophilus thermoluteolus
MKRRDFLKAVTAAVALPEAFVSLPSFA

SEQ ID NO: 42 - DNA, 81 bp, Hydrogenophilus thermoluteolus
  source 1..81: mol_type = genomic DNA
atgaaaagaagggattttctcaaggcggtgactgctgccgttgctcttccggaggcattcgtctccctgcccagcttcgct

SEQ ID NO: 43 - protein, 25 aa, Hydrogenophilus thermoluteolus
MKQFKPFVYGAAAALAFALTPQAHA

SEQ ID NO: 44 - DNA, 75 bp, Hydrogenophilus thermoluteolus
  source 1..75: mol_type = genomic DNA
atgaagcagttcaaaccattcgtatacggggcggctgcggcactggcgttcgcgctgacgccgcaagcccatgcc

SEQ ID NO: 45 - protein, 40 aa, Hydrogenophilus thermoluteolus
MATVREPTTASTPLRPRRNLLRALGALFVTTATAPFPVRS

SEQ ID NO: 46 - DNA, 120 bp, Hydrogenophilus thermoluteolus
  source 1..120: mol_type = genomic DNA
atggccactgttcgcgaaccgacgactgcatccactcccctccggccccgccgcaacctcctgcgcgcgctgggtgcactgttcgtgaccacggccacggcaccctttccggtgcgttcg

SEQ ID NO: 47 - protein, 22 aa, Hydrogenophilus thermoluteolus
MRAIRWGMVIALSLANLSPAWA

SEQ ID NO: 48 - DNA, 66 bp, Hydrogenophilus thermoluteolus
  source 1..66: mol_type = genomic DNA
atgcgcgcgatacggtggggaatggtcatcgcactctcgttggcgaacctgtcgcctgcgtgggcg

SEQ ID NO: 49 - protein, 20 aa, Hydrogenophilus thermoluteolus
MQKKLIALAVAGLVAAPAMA

SEQ ID NO: 50 - DNA, 60 bp, Hydrogenophilus thermoluteolus
  source 1..60: mol_type = genomic DNA
atgcaaaagaaactgatcgctctggcagttgccgggctggtcgctgcgccggcgatggct

SEQ ID NO: 51 - protein, 21 aa, Hydrogenophilus thermoluteolus
MKKVTFALAGVMGFSATLAWA

SEQ ID NO: 52 - DNA, 63 bp, Hydrogenophilus thermoluteolus
  source 1..63: mol_type = genomic DNA
atgaaaaaggtaacgttcgcgctcgctggtgtgatggggttttcggctaccctggcatgggca

SEQ ID NO: 53 - protein, 23 aa, Hydrogenophilus thermoluteolus
MKKIAQLLVVAGVMTVGAAPAFA

SEQ ID NO: 54 - DNA, 69 bp, Hydrogenophilus thermoluteolus
  source 1..69: mol_type = genomic DNA
atgaaaaaaatcgcacaactgttggtggtggccggggtgatgacggttggagccgcaccggcgttcgcc

SEQ ID NO: 55 - protein, 46 aa, Hydrogenophilus thermoluteolus
MEEKIMTLTKTTANEPQSISRRKALKTLGKLTATSLAAAHAPWVHA

SEQ ID NO: 56 - DNA, 138 bp, Hydrogenophilus thermoluteolus
  source 1..138: mol_type = genomic DNA
atggaggagaaaattatgacactaactaagacaactgctaacgaaccgcagtcgatttcgcgtagaaaagccctcaaaacgttgggaaaactgacggccaccagccttgcggctgcgcatgccccttgggttcacgct

SEQ ID NO: 57 - protein, 34 aa, Hydrogenophilus thermoluteolus
MFERRAGRTVAPRRIARWWCAFALLLCTAGVAFA

SEQ ID NO: 58 - DNA, 102 bp, Hydrogenophilus thermoluteolus
  source 1..102: mol_type = genomic DNA
atgttcgaacggcgtgccgggcgcacggtggcaccgcgccgcattgcgcggtggtggtgcgcctttgcactgttgctctgcaccgccggggttgcgttcgca

SEQ ID NO: 59 - protein, 24 aa, Hydrogenophilus thermoluteolus
MVGMMRTLACLMMLWWLGIQVAMA

SEQ ID NO: 60 - DNA, 72 bp, Hydrogenophilus thermoluteolus
  source 1..72: mol_type = genomic DNA
atggtcggcatgatgcgcactctggcctgtttgatgatgctttggtggctgggcattcaggtcgctatggct

SEQ ID NO: 61 - protein, 24 aa, Hydrogenophilus thermoluteolus
MTLRALLTLLSTALPLAYAPFAVA

SEQ ID NO: 62 - DNA, 72 bp, Hydrogenophilus thermoluteolus
  source 1..72: mol_type = genomic DNA
atgacgcttcgcgcgctcttgactttgttatcgactgctctgcccttggcgtacgccccgtttgctgtagcg

SEQ ID NO: 63 - protein, 22 aa, Hydrogenophilus thermoluteolus
MRERIAMRVGLWATVAMVVLAG

SEQ ID NO: 64 - DNA, 66 bp, Hydrogenophilus thermoluteolus
  source 1..66: mol_type = genomic DNA
atgagggaacggattgcgatgcgagtcggattgtgggcgacggtggcgatggtcgtgctcgctggg

SEQ ID NO: 65 - protein, 25 aa, Hydrogenophilus thermoluteolus
MNKRAFVHTLLATVALGAWVPTVRA

SEQ ID NO: 66 - DNA, 75 bp, Hydrogenophilus thermoluteolus
  source 1..75: mol_type = genomic DNA
atgaacaaaagagcctttgtgcatacgttgcttgctactgttgcgcttggcgcgtgggttccaacggtccgcgcc

SEQ ID NO: 67 - protein, 39 aa, Hydrogenophilus thermoluteolus
MSAPRIAHSRLFPRRLHHWLTTVALALLVGFGLTTPVRA

SEQ ID NO: 68 - DNA, 117 bp, Hydrogenophilus thermoluteolus
  source 1..117: mol_type = genomic DNA
atgagtgccccccggattgcccattcacgcctgttcccacgccgtctgcaccattggctgaccacggtggctttggccctgctcgtggggtttggtttgaccacgccggttcgggcc

SEQ ID NO: 69 - protein, 22 aa, Hydrogenophilus thermoluteolus
MRLGIRGWIAVGLFATATLAQA

SEQ ID NO: 70 - DNA, 66 bp, Hydrogenophilus thermoluteolus
  source 1..66: mol_type = genomic DNA
atgcgcctaggaattcgcggatggattgcagttggcttgttcgctacggctacgttggcacaggcc

SEQ ID NO: 71 - protein, 9 aa, Hydrogenophilus thermoluteolus
MAFKRAQTG

SEQ ID NO: 72 - DNA, 27 bp, Hydrogenophilus thermoluteolus
  source 1..27: mol_type = genomic DNA
atggctttcaaacgtgcgcaaacgggt

SEQ ID NO: 73 - protein, 40 aa, Hydrogenophilus thermoluteolus
MKRDSGSIDWRRRRLIKGAVAASLLAGVGGYWHEEIRAFA

SEQ ID NO: 74 - DNA, 120 bp, Hydrogenophilus thermoluteolus
  source 1..120: mol_type = genomic DNA
atgaaacgcgacagcggttcgatcgattggcgtcgccgtcggctgatcaaaggagcggttgctgcttcgctcctggcaggcgttggcggttattggcacgaggaaatccgtgcgtttgcc

SEQ ID NO: 75 - protein, 23 aa, Hydrogenophilus thermoluteolus
MRRWVTRIAMGLLFCAITPALQA

SEQ ID NO: 76 - DNA, 69 bp, Hydrogenophilus thermoluteolus
  source 1..69: mol_type = genomic DNA
atgaggcgctgggtgacgcgaatcgcgatggggctgttgttctgtgcgatcacaccagcgcttcaggcg

SEQ ID NO: 77 - protein, 20 aa, Hydrogenophilus thermoluteolus
MGLHLRQWMVVMVAPAVLAA

SEQ ID NO: 78 - DNA, 60 bp, Hydrogenophilus thermoluteolus
  source 1..60: mol_type = genomic DNA
atgggtcttcatctgcgccagtggatggtggttatggttgcaccggccgttttggcagcc

SEQ ID NO: 79 - protein, 25 aa, Hydrogenophilus thermoluteolus
MTRFLTTRTARAGAAVLASAALLAG

SEQ ID NO: 80 - DNA, 75 bp, Hydrogenophilus thermoluteolus
  source 1..75: mol_type = genomic DNA
atgacccgatttttgaccacccgtaccgcgcgtgctggagcagccgtgctcgcgtcggcagcgttgcttgccggt

SEQ ID NO: 81 - protein, 25 aa, Hydrogenophilus thermoluteolus
MKRRWQQAVMAVAFSLASLSVMAQA

SEQ ID NO: 82 - DNA, 75 bp, Hydrogenophilus thermoluteolus
  source 1..75: mol_type = genomic DNA
atgaaacgtcgttggcagcaagccgtaatggcggtggcattttcgctcgcgagcctttcggtgatggcgcaagcc

SEQ ID NO: 83 - protein, 30 aa, Hydrogenophilus thermoluteolus
MSAIALLRPKKGRHLLLILGFVATNPLAVA

SEQ ID NO: 84 - DNA, 90 bp, Hydrogenophilus thermoluteolus
  source 1..90: mol_type = genomic DNA
atgtcggcaatcgctcttttgcgcccgaaaaaggggcgtcatctgcttttgatccttggattcgtcgcgacaaacccacttgccgttgcc

SEQ ID NO: 85 - protein, 24 aa, Hydrogenophilus thermoluteolus
MRKASKLAFAVSCMTMAMSGIAHA

SEQ ID NO: 86 - DNA, 72 bp, Hydrogenophilus thermoluteolus
  source 1..72: mol_type = genomic DNA
atgagaaaggcaagcaaactcgcattcgcagtttcatgcatgacgatggcaatgagcggcattgctcatgca

SEQ ID NO: 87 - protein, 20 aa, Hydrogenophilus thermoluteolus
MWAGALFFCLLGVVGTRAVA

SEQ ID NO: 88 - DNA, 60 bp, Hydrogenophilus thermoluteolus
  source 1..60: mol_type = genomic DNA
atgtgggccggtgcgctcttcttttgccttctgggcgtagtggggacgcgcgcggtggcc

SEQ ID NO: 89 - protein, 28 aa, Hydrogenophilus thermoluteolus
MMARSFLKAWFPRLLVLLLSLPLVVARA

SEQ ID NO: 90 - DNA, 84 bp, Hydrogenophilus thermoluteolus
  source 1..84: mol_type = genomic DNA
atgatggcgcgttcgttcctgaaagcgtggtttccaaggttgttggtgctcttattgtcactgccgctcgtcgtggcgcgtgcg

SEQ ID NO: 91 - protein, 26 aa, Hydrogenophilus thermoluteolus
MKKRVGIWVIRWVLASVMVALPPAWA

SEQ ID NO: 92 - DNA, 78 bp, Hydrogenophilus thermoluteolus
  source 1..78: mol_type = genomic DNA
atgaaaaaaagggtaggtatctgggtgatccgatgggttttggcgagcgtcatggtcgcgcttccgcctgcgtgggct

SEQ ID NO: 93 - protein, 26 aa, Hydrogenophilus thermoluteolus
MERLLRRRVVGIAAAALTGLSFPAWS

SEQ ID NO: 94 - DNA, 78 bp, Hydrogenophilus thermoluteolus
  source 1..78: mol_type = genomic DNA
atggagcgtttactccgacgtcgcgtggtgggtattgcagcggcggctttgaccggtctgagcttcccggcatggtcc

SEQ ID NO: 95 - protein, 28 aa, Hydrogenophilus thermoluteolus
MARKQIARTTLTSLLVSGLVATAMTSWA

SEQ ID NO: 96 - DNA, 84 bp, Hydrogenophilus thermoluteolus
  source 1..84: mol_type = genomic DNA
atggcacgcaagcaaatcgcacgtacgactctgacatcccttctggtttctggccttgtcgccaccgcaatgaccagctgggca

SEQ ID NO: 97 - protein, 28 aa, Hydrogenophilus thermoluteolus
MRRWEGKRIIVTWMACLAPFFASVGATA

SEQ ID NO: 98 - DNA, 84 bp, Hydrogenophilus thermoluteolus
  source 1..84: mol_type = genomic DNA
atgagacgctgggagggaaaacgcatcatcgtaacctggatggcgtgcctcgcgccattcttcgcatcagtcggtgcgacggcg

SEQ ID NO: 99 - protein, 45 aa, Hydrogenophilus thermoluteolus
MTKPTRTDPRPTQNAVTGERAPDRRRRLALTAPAALALAAGGARA

SEQ ID NO: 100 - DNA, 135 bp, Hydrogenophilus thermoluteolus
  source 1..135: mol_type = genomic DNA
atgaccaaacccacgcgaaccgacccaagacccacccaaaacgccgtgacgggcgaacgcgcgcccgaccgtcgccgtcgactggcactgaccgcaccggctgcgttggcgctcgcagccgggggggcacgggcg

SEQ ID NO: 101 - protein, 43 aa, Hydrogenophilus thermoluteolus
MRSKQDGKLTTLIGRRTFMKRGAAVAATLFGLSAGLVRTPAQA

SEQ ID NO: 102 - DNA, 129 bp, Hydrogenophilus thermoluteolus
  source 1..129: mol_type = genomic DNA
atgcgcagcaagcaagacgggaaattgaccactctgatcggccggagaaccttcatgaaaagaggggccgccgtggctgcaacgctctttggcctttccgctgggctcgtgcgcacaccggcacaggcc

SEQ ID NO: 103 - protein, 20 aa, Hydrogenophilus thermoluteolus
MRLAALTYIAALVATPGAAA

SEQ ID NO: 104 - DNA, 60 bp, Hydrogenophilus thermoluteolus
  source 1..60: mol_type = genomic DNA
atgcgacttgccgcgctgacgtacatagctgctctggtggcgacacccggtgcggctgcc

SEQ ID NO: 105 - protein, 21 aa, Hydrogenophilus thermoluteolus
MKKTTLLLTLGLAVLTPTLSG

SEQ ID NO: 106 - DNA, 63 bp, Hydrogenophilus thermoluteolus
  source 1..63: mol_type = genomic DNA
atgaaaaaaacgaccctgttgctcaccctggggttggcggtgctcacccccacgttgtcgggc

SEQ ID NO: 107 - protein, 42 aa, Hydrogenophilus thermoluteolus
MKNDPAINPDMAAAPFSRRTALKALFAQAVGLSFPLPGHSSV

SEQ ID NO: 108 - DNA, 126 bp, Hydrogenophilus thermoluteolus
  source 1..126: mol_type = genomic DNA
atgaaaaatgatcctgcaatcaatcccgatatggctgccgccccattttcccgacgcaccgccctcaaagcgctctttgcgcaagcggtcggtttgtcgttcccgttgcccggtcacagctccgtg

SEQ ID NO: 109 - protein, 20 aa, Hydrogenophilus thermoluteolus
MKRVLFLGLLCLGFHAMAFA

SEQ ID NO: 110 - DNA, 60 bp, Hydrogenophilus thermoluteolus
  source 1..60: mol_type = genomic DNA
atgaaaagggtactgttcttgggtttgctctgccttgggtttcacgcgatggcgttcgcc

SEQ ID NO: 111 - protein, 26 aa, Hydrogenophilus thermoluteolus
MNPNHRKIFHLGIALMSLLTPMASHS

SEQ ID NO: 112 - DNA, 78 bp, Hydrogenophilus thermoluteolus
  source 1..78: mol_type = genomic DNA
atgaatccgaaccaccgcaaaatttttcacctaggaatcgcgctcatgagtctccttaccccgatggcttcgcactcg

SEQ ID NO: 113 - protein, 24 aa, Hydrogenophilus thermoluteolus
MVTWSRRRWLAAALTMGMVSRSWG

SEQ ID NO: 114 - DNA, 72 bp, Hydrogenophilus thermoluteolus
  source 1..72: mol_type = genomic DNA
atggttacttggagcagacgccggtggttggccgcagctttgaccatggggatggtgtcgcgaagctggggc

SEQ ID NO: 115 - protein, 27 aa, Hydrogenophilus thermoluteolus
MTTKWVMVGPRWLLAVVLIMSAAVARG

SEQ ID NO: 116 - DNA, 81 bp, Hydrogenophilus thermoluteolus
  source 1..81: mol_type = genomic DNA
atgacgacgaaatgggtgatggtgggaccccgatggttgctggcggtggtgctgatcatgagcgctgccgtggctaggggg

SEQ ID NO: 117 - protein, 22 aa, Hydrogenophilus thermoluteolus
MSVFRLRKGFMALVAVTLILTG

SEQ ID NO: 118 - DNA, 66 bp, Hydrogenophilus thermoluteolus
  source 1..66: mol_type = genomic DNA
atgtcggtttttcggctgcgcaaagggttcatggcactggttgcagtaaccctgatcctcacggga

SEQ ID NO: 119 - protein, 40 aa, Hydrogenophilus thermoluteolus
MYRNEHDRGAPTRRHFLAYCAQWLGALATLPLANPSRAQA

SEQ ID NO: 120 - DNA, 120 bp, Hydrogenophilus thermoluteolus
  source 1..120: mol_type = genomic DNA
atgtatagaaacgaacacgaccgcggcgcccccacgcgccgccattttctcgcctattgtgcgcagtggttgggcgcgctggcaaccctgccgcttgcgaacccatcgcgcgcacaagcc

SEQ ID NO: 121 - protein, 19 aa, Hydrogenophilus thermoluteolus
MKPLVVASSLLLVAGAAHA

SEQ ID NO: 122 - DNA, 57 bp, Hydrogenophilus thermoluteolus
  source 1..57: mol_type = genomic DNA
atgaaaccactcgtagtcgctagctcgctgcttctcgtcgctggcgccgcgcacgct

SEQ ID NO: 123 - protein, 25 aa, Hydrogenophilus thermoluteolus
MKRNTFRLTTLASALFVAGLSSAHA

SEQ ID NO: 124 - DNA, 75 bp, Hydrogenophilus thermoluteolus
  source 1..75: mol_type = genomic DNA
atgaaaagaaatacgtttcgtttgacgacgcttgccagcgcgctttttgttgcaggtctttcttcggcgcacgcc

SEQ ID NO: 125 - protein, 20 aa, Hydrogenophilus thermoluteolus
MKTLTLALLALPWATSVAFA

SEQ ID NO: 126 - DNA, 60 bp, Hydrogenophilus thermoluteolus
  source 1..60: mol_type = genomic DNA
atgaagaccttgacattggcactgctggcgctgccttgggcaaccagtgtcgcgtttgcg

SEQ ID NO: 127 - protein, 18 aa, Hydrogenophilus thermoluteolus
MNVVRLVGMVTAAMVLAA

SEQ ID NO: 128 - DNA, 54 bp, Hydrogenophilus thermoluteolus
  source 1..54: mol_type = genomic DNA
atgaatgtcgtgcgactggttgggatggtgacggctgcgatggtgttggctgcg

SEQ ID NO: 129 - protein, 22 aa, Hydrogenophilus thermoluteolus
MKRFALVRRWLVCAALVVGISG

SEQ ID NO: 130 - DNA, 66 bp, Hydrogenophilus thermoluteolus
  source 1..66: mol_type = genomic DNA
atgaaacgtttcgcgcttgtacggcgttggctggtgtgcgctgcgctggtggttgggatttcgggg

SEQ ID NO: 131 - protein, 18 aa, Hydrogenophilus thermoluteolus
MKWRQVVCGVAAAFALAG

SEQ ID NO: 132 - DNA, 54 bp, Hydrogenophilus thermoluteolus
  source 1..54: mol_type = genomic DNA
atgaagtggagacaggtcgtttgtggggtcgcagcagcgttcgcgcttgcgggg

SEQ ID NO: 133 - protein, 57 aa, Hydrogenophilus thermoluteolus
MTEELRNRIGLIRKAPENFLTPEEIEAIKKGRRDFIRKAFATATALAASGPVINAYG

SEQ ID NO: 134 - DNA, 171 bp, Hydrogenophilus thermoluteolus
  source 1..171: mol_type = genomic DNA
atgaccgaagaactgcgaaaccgaatcggcctgattcgtaaggcgccggagaattttttgacgccggaagagatcgaggccatcaagaaggggcggcgcgatttcattcgcaaagcgtttgccacggcaaccgcgttggccgcgagcggaccggtgatcaacgcctacgga

SEQ ID NO: 135 - protein, 25 aa, Hydrogenophilus thermoluteolus
MKNRKRQIGIAVASALAIFSGGVHA

SEQ ID NO: 136 - DNA, 75 bp, Hydrogenophilus thermoluteolus
  source 1..75: mol_type = genomic DNA
atgaaaaacaggaaacggcaaatcgggatcgcggtggcgtcggcgctcgcgatcttttcgggtggtgtccatgcc

SEQ ID NO: 137 - protein, 42 aa, Hydrogenophilus thermoluteolus
METFYEVMRRQGITRRSFLKFCSLTATALGLGPSAVPRIVHA

SEQ ID NO: 138 - DNA, 126 bp, Hydrogenophilus thermoluteolus
  source 1..126: mol_type = genomic DNA
atggaaaccttttacgaagtgatgcggcgccaggggatcacacggcgcagttttctcaagttttgtagcctcaccgccacggcgctggggctcgggcccagtgcggtgccgcgcatcgtccatgcg

SEQ ID NO: 139 - protein, 22 aa, Hydrogenophilus thermoluteolus
MRWNHRNRTAAFLLVSAALVSG

SEQ ID NO: 140 - DNA, 66 bp, Hydrogenophilus thermoluteolus
  source 1..66: mol_type = genomic DNA
atgcgctggaaccaccgcaatcgaaccgctgccttcctcttggtgagcgctgcgctggtaagcggt

SEQ ID NO: 141 - protein, 23 aa, Hydrogenophilus thermoluteolus
MKSRLAVLFLGVSLAFNGIAVQA

SEQ ID NO: 142 - DNA, 69 bp, Hydrogenophilus thermoluteolus
  source 1..69: mol_type = genomic DNA
atgaaaagtcgtctggctgtcttgtttcttggtgtaagcttggcattcaatgggatcgccgttcaggcg

SEQ ID NO: 143 - protein, 11 aa, Hydrogenophilus thermoluteolus
MLFLIVSPAFA

SEQ ID NO: 144 - DNA, 33 bp, Hydrogenophilus thermoluteolus
  source 1..33: mol_type = genomic DNA
atgctttttttgattgtatcacccgcgttcgcc

SEQ ID NO: 145 - protein, 23 aa, Hydrogenophilus thermoluteolus
MVRKVGIGCALWLIAAQWAYGSA

SEQ ID NO: 146 - DNA, 69 bp, Hydrogenophilus thermoluteolus
  source 1..69: mol_type = genomic DNA
atggttcgaaaagtggggattgggtgcgccttgtggctcatcgcggcccagtgggcttacggatcggct

SEQ ID NO: 147 - protein, 30 aa, Hydrogenophilus thermoluteolus
MSTLVCSHLRPLALTALTALIVALPGPLYA

SEQ ID NO: 148 - DNA, 90 bp, Hydrogenophilus thermoluteolus
  source 1..90: mol_type = genomic DNA
atgagcacgcttgtctgcagccatttacgcccgctcgcgttgaccgcactcacagcgctgatcgtggcattgcccggaccactctacgcg

SEQ ID NO: 149 - protein, 30 aa, Hydrogenophilus thermoluteolus
MEMTRFVVRRNLLAWLVVGAVAGVTATAHA

SEQ ID NO: 150 - DNA, 90 bp, Hydrogenophilus thermoluteolus
  source 1..90: mol_type = genomic DNA
atggaaatgacacgttttgtggttcgccgtaatctgttggcttggctggtggttggcgcagtggctggggtgaccgccacggcacacgca

SEQ ID NO: 151 - protein, 23 aa, Hydrogenophilus thermoluteolus
MKRVALLLQATLLFFGGALGTHA

SEQ ID NO: 152 - DNA, 69 bp, Hydrogenophilus thermoluteolus
  source 1..69: mol_type = genomic DNA
atgaaacgggttgccctactcctgcaagcaacccttttgtttttcgggggtgcgcttgggacacacgcg

SEQ ID NO: 153 - DNA, 35 bp, synthetic construct
  source 1..35: mol_type = other DNA
ttttataacccgggccatcgactgcacggtgcacc

SEQ ID NO: 154 - DNA, 35 bp, synthetic construct
  source 1..35: mol_type = other DNA
tgctagcactgtttcctgtgtgaaattgttatccg

SEQ ID NO: 155 - DNA, 38 bp, synthetic construct
  source 1..38: mol_type = other DNA
ggaaacagtgctagcagatctggaggagaaacgcatat

SEQ ID NO: 156 - DNA, 72 bp, synthetic construct
  source 1..72: mol_type = other DNA
cagtgcggccgcaagcttgtcgacggagctcgaattcggatccgatatcagcatatgcgtttctcctccaga

SEQ ID NO: 157 - DNA, 80 bp, synthetic construct
  source 1..80: mol_type = other DNA
acaagcttgcggccgcactgcagcaccatcaccaccatcattgataagatccggctgctaacaaagcccgaaaggaagct

SEQ ID NO: 158 - DNA, 63 bp, synthetic construct
  source 1..63: mol_type = other DNA
tatttgaatcgagttattgctcagcggtggcagcagccaactcagcttcctttcgggctttgt

SEQ ID NO: 159 - DNA, 35 bp, synthetic construct
  source 1..35: mol_type = other DNA
taactcgattcaaataaaacgaaaggctcagtcga

SEQ ID NO: 160 - DNA, 35 bp, synthetic construct
  source 1..35: mol_type = other DNA
cctagatccgcggagtttgtagaaacgcaaaaagg

SEQ ID NO: 161 - DNA, 35 bp, synthetic construct
  source 1..35: mol_type = other DNA
acaaactccgcggatctaggtgaagatcctttttg

SEQ ID NO: 162 - DNA, 35 bp, synthetic construct
  source 1..35: mol_type = other DNA
cgtccgcggccagcaaaaggccaggaaccgtaaaa

SEQ ID NO: 163 - DNA, 35 bp, synthetic construct
  source 1..35: mol_type = other DNA
ttgctggccgcggacgtagaaagcctgtccgcaga

SEQ ID NO: 164 - DNA, 35 bp, synthetic construct
  source 1..35: mol_type = other DNA
ggcccgggttataaaagccagtcattaggcctatc

SEQ ID NO: 165 - DNA, 35 bp, synthetic construct
  source 1..35: mol_type = other DNA
aattgtcagataggcctaatgactggcttttataa

SEQ ID NO: 166 - DNA, 35 bp, synthetic construct
  source 1..35: mol_type = other DNA
tgacgccagaagcattggtgcaccgtgcagtcgat

SEQ ID NO: 167 - DNA, 19 bp, synthetic construct
  source 1..19: mol_type = other DNA
gatctggaggagaaacgca

SEQ ID NO: 168 - DNA, 17 bp, synthetic construct
  source 1..17: mol_type = other DNA
tatgcgtttctcctcca

SEQ ID NO: 169 - DNA, 35 bp, synthetic construct
  source 1..35: mol_type = other DNA
gaggccatctaggccatgagtaagtctgacggaac

SEQ ID NO: 170 - DNA, 35 bp, synthetic construct
  source 1..35: mol_type = other DNA
atccggcacccatatctgaaccggacgcaaacccg

SEQ ID NO: 171 - DNA, 35 bp, synthetic construct
  source 1..35: mol_type = other DNA
ttcagatatgggtgccggatacccgccgcccgggc

SEQ ID NO: 172 - DNA, 35 bp, synthetic construct
  source 1..35: mol_type = other DNA
aaggccttcatggccttatttcgcgattcccaaga

SEQ ID NO: 173 - DNA, 87 bp, synthetic construct
  source 1..87: mol_type = other DNA
gcatatggaacgtcgtcgtttcctcaaaggcgccggccttgccggcattctggctgccggcacggcgcctgcgatcatccatgcaca

SEQ ID NO: 174 - DNA, 87 bp, synthetic construct
  source 1..87: mol_type = other DNA
cgactgtgcatggatgatcgcaggcgccgtgccggcagccagaatgccggcaaggccggcgcctttgaggaaacgacgacgttccat

SEQ ID NO: 175 - DNA, 34 bp, synthetic construct
  source 1..34: mol_type = other DNA
ggctacggtctcaattcgagctccgtcgacaagc

SEQ ID NO: 176 - DNA, 36 bp, synthetic construct
  source 1..36: mol_type = other DNA
ggctacggtctcgcatatgcgtttctcctccagatc

SEQ ID NO: 177 - DNA, 11 bp, synthetic construct
  source 1..11: mol_type = other DNA
gcgggtctcat

SEQ ID NO: 178 - DNA, 16 bp, synthetic construct
  source 1..16: mol_type = other DNA
gaattcggagacccgc

SEQ ID NO: 179 - DNA, 744 bp, synthetic construct
  source 1..744: mol_type = other DNA
gcgggtctcatatgtcgaaaggcgaagaactcttcaccggcgtcgtcccgatcctcgtcgaactcgacggcgacgtcaacggccacaaattctcggtccgcggcgaaggcgaaggcgacgcgaccaacggcaaactcaccctcaaattcatctgcaccaccggcaaactcccggtcccgtggccgaccctcgtcaccaccctcacctacggcgtcctctgcttctcgcgctacccggaccacatgaaacgccacgacttcttcaaatcggcgatgccggaaggctacgtccaggaacgcaccatctcgttcaaagacgacggcacctacaaaacccgcgcggaagtcaaattcgaaggcgacaccctcgtcaaccgcatcgaactcaaaggcatcgacttcaaagaagacggcaacatcctcggccacaaactcgaatacaacttcaactcgcacaacgtctacatcaccgcggacaaacagaaaaacggcatcaaagcgtacttcaaaatccgccacaacgtcgaagacggctcggtccagctcgcggaccactaccagcagaacaccccgatcggcgacggcccggtcctcctcccggacaaccactacctctcgacccagtcggtcctctcgaaagacccgaacgaaaaacgcgaccacatggtcctcctcgaagacgtcaccgcggcgggcatcacccacggcatggacgaactctacaaataagaattcggagacccgc

SEQ ID NO: 180 - DNA, 35 bp, synthetic construct
  source 1..35: mol_type = other DNA
ggctacggtctcagtcgaaaggcgaagaactcttc

SEQ ID NO: 181 - DNA, 33 bp, synthetic construct
  source 1..33: mol_type = other DNA
ggctacggtctcgatgcgtttctcctccagatc